European Patent Application EP 4 779 311 A2, published July 22, 2026. Title: SELECTING A PATIENT HAVING AN ELEVATED NECTIN-4. Applicant: BicycleTx Limited. Application EP, filed August 17, 2021. The sequence listing filed with the application follows.

SEQUENCE LISTING (1 sequence)

SEQ ID NO: 1 - protein, 26 aa, Synthetic construct
  MOD_RES 1: note = B-Ala
  SITE 2..11: note = sarcosine
  MOD_RES 14: note = 1-napthylalanine
  MOD_RES 15: note = d-aspartic acid
  MOD_RES 18: note = homoarginine
  MOD_RES 24: note = hydroxyproline
AXXXXXXXXXXCPADCMRDWSTPPWC